European Patent Specification EP 3 488 015 B1, published February 21, 2024. Title: HIGHLY POLYMORPHIC AND MODULAR EXTRAGENIC (H.P.M.E.) MARKERS WITHIN SPECIFIC TAXA OF MICROORGANISMS AND USE THEREOF FOR THEIR DIFFERENTIATION, IDENTIFICATION AND QUANTIFICATION. Applicant: MICROBION S.R.L. The sequence listing filed with the application follows.

SEQUENCE LISTING (81 sequences)

SEQ ID NO: 1 - DNA, 1087 bp, Oenococcus alcolitolerans
tgatcgatctcgtcgtgagcggccaaaatctgcgtaaggatcctttctgtgtacttttcgaggatcttaccggctttcgtcaattgaacgcggccatgcgaatgattcctggtaactaattcttgtttaaattctttttccaatcgctggatggcataagaaatagttggttggctgacattgaaaaaagctgccgtttgtgaaaacgactccactttggccaggcgctgaaaatactctaaatcagtgaatttcatataaatttattttatctcttttgcagcttttgactatatcagctgcgataaaatatcctgaatctgtttgtttattaggagagagaaatgacagatccagtagatattttaaacgatccctttaaaaacaaaggaaccgcttttactcaagaagaacgcaaagcactgggcttgcagggacttttgccctcatgtgtgcaaactattgatcagcaagctgcacaagcctatgctcaatttcaaagcaaagctgataatctagaaaaaagacttttcttgatggaacttttcaacaccaaccacgtgctgttctataagcttttttcacaacacgtcgttgaattcatgccgatcgtctatgatccgactatcgctgatacgattgaaaattattctgaacttttcgttgaaacacagggagctgcttttttggatatccagcatccagaaaacatcgaagccagtttgaaaaatgccgctgacggtcgtgacataaaattgatcgtcgtcactgatgctgagggcattttaggtatcggcgactggggtgttcaaggggtcgatatcgccgttggaaaattgatggtctacaccgtggctgcaggacttgatccaaagagtgtcttgccggtcgtgatcgatgccggaaccaataatcaaaaacttttaaacgatcctttgtatttaggaaaccgttttaaccgtgttcgcggtcaagcttatgatgattttatcgatacttttgttgaaaaatcggaaaatctttttccagatatgtatttgcattgggaagactttgggcgtttgaatgccgcaaatatttgaataga

SEQ ID NO: 2 - DNA, 788 bp, Lactobacillus brevis
ccatacagagccgccctcaacagtttgcagtccttccagcagattctcagcctgcaatcgtgcggcaattcgtggaaaataataattttcgataattggtggcaaccccagcgtggtttggcgagcagctaaatgggctagttcttggtgggctagcgttaattcactgaggacgacttgggcgtgaatggctaattgctcaccgctcggggtaatttgaatatcattgtgtacccgatcccggatgactaatttggtttcaaattcggtctctaatcgtttgatagccgtggtgatcgtgggctgagtcacaccgaaraaggctgctaccttagaaaaatttttttgtagaataagctgctggaaataatccaaatcttttgtattcatattttctcctgtcaaatcaaggctgattactacattataaaataattttataacaatcgctacgtttgactataaaattttcagggcgttatagtgcaatatgtaaataagagctatccaaattggaggaaaatcatgatgacgcaaacagcagatacgattttaaataaccccttcttaaataaaggaaccgcgttcacacaagcagaacggcgggaacttggcttggttgggacattgccagcccaagttcaaacgattgatgaacaagccactcaggcctatgcccaataccaaagcaagccaagtgacctggaaaagcggattttcttaatgaatctctttaacgaaaaccggacattattcttccatttaatggatgaacacgtggttgaatt

SEQ ID NO: 3 - DNA, 788 bp, Lactobacillus brevis
ccatacagagccgccctcaacagtttgcagtccttccagcagattctcagcctgcaatcgtgcggcaattcgtggaaaataataattttcgataattggtggcaaccccagcgtggtttggcgagcagctaaatgggctagttcttggtgggctagcgttaattcactgaggacgacttgggcgtgaatggctaattgctcaccgctcggggtaatttgaatatcattgtgtacccgatcccggatgactaatttggtttcaaattcggtctctaatcgtttgatagccgtggtgatcgtgggctgagtcacaccgaagaaggctgctaccttagaaaaatttttttgtagaataagctgctggaaataatccaaatcttttgtattcatattttctcctgtcaaatcaaggctgattactacattataaaataattttataacaatcgctacgtttgactataaaattttcagggcgttatagtgcaatatgtaaataagagctatccaaattggaggaaaatcatgatgacgcaaacagcagatacgattttaaataaccccttcttaaataaaggaaccgcgttcacacaagcagaacggcgggaacttggcttggttgggacattgccagcccaagttcaaacgattgatgaacaagccactcaggcctatgcccaataccaaagcaagccaagtgacctggaaaagcggattttcttaatgaatctctttaacgaaaaccggacattattcttccatttaatggatgaacacgtggttgaatt

SEQ ID NO: 4 - DNA, 788 bp, Lactobacillus brevis
ccatacagagccgccctcgacagtttgcagtccttccagcagattctcagcctgcaatcgtgcggcaattcgtggaaaataataattttcgataattggtggcaaccccagcgtggtttggcgagcagctaaatgtgctagttcttggtgggctagcgttaattcactgaggacgacttgggcgtgaatggctagttgctcaccgctcggggtaatttgaatatcattgtgtacccgatcccggatgactaatttggtttcaaattcggtctctaatcgtttgatagccgtggtgatcgtgggctgagtcacaccgaagaaggttgctaccttagaaaaatttttttgtagaataagctgctggaaataatccaaatattttgtattcatattttctcctgtcaaatcaaggctgattgctacattataaaataattttataacaatcgctacatttgactataaaatttccagggcgttatagtgcaatatgtaaataagagctatccaaattggaggaaaatcatgatgacgcaaacagcagatacgattttaaataaccccttcttaaataaaggaaccgcgttcacacaagcagaacggcgggaacttggcttggttgggacattgccagcccaagttcaaacgattgatgaacaagccactcaggcctatgcccaataccaaagcaagccaagtgacctggaaaagcggattttcttaatgaatctctttaacgaaaaccggacattattcttccatttaatggatgaacacgtggttgaatt

SEQ ID NO: 5 - DNA, 788 bp, Lactobacillus brevis
ccatacagagccgccctcaacagtttgcagtccttccagcagattctcagcctgcaatcgtgcggcaattcgtggaaaataataattttcgataattggtggcaaccccagcgtggtttggcgagcagctaaatgggctagttcttggtgggctagcgttaattcactgaggacgacttgggcgtgaatggctaattgctcaccgctcggggtaatttgaatatcattgtgtacccgatcccggatgactaatttggtttcaaattcggtctctaatcgtttgatagccgtggtgatcgtgggctgagtcacaccgaagaaggctgctaccttagaaaaatttttttgtagaataagctgctggaaataatccaaatcttttgtattcatattttctcctgtcaaatcaaggctgattactacattataaaataattttataacaatcgctacgtttgactataaaattttcagggcgttatagtgcaatatgtaaataagagctatccaaattggaggaaaatcatgatgacgcaaacagcagatacgattttaaataaccccttcttaaataaaggaaccgcgttcacacaagcagaacggcgggaacttggcttggttgggacattgccagcccaagttcaaacgattgatgaacaagccactcaggcctatgcccaataccaaagcaagccaagtgacctggagaagcggattttcttaatgaatctctttaacgaaaaccggacattattcttccatttaatggatgaacacgtggttgaatt

SEQ ID NO: 6 - DNA, 788 bp, Lactobacillus brevis
ccatacagagccaccctcaaccgtttgcagtccttccagcagattctcagcctgcaatcgtgcggcaattcgtggaaaataataattttcgataattggtggcaaccccagcgtggtttggcgagcagctaaatgtgctagttcttggtgggctagcgttaattcactgaggacgacttgggcgtgaatggctagttgctcaccgctcggggtaatttgaatatcattgtgtacccgatcccggatgactaatttggtttcaaattcggtctctaatcgtttgatagccgtggtgatcgtgggctgagtcacaccgaagaaggttgctaccttagaaaaatttttttgtagaataagctgctggaaataatccaaatcttttgtattcatattttctcctgtcaaatcaaggctgattgctacattataaaataattttataacaatcgctacatttgactataaaatttccagggcgttatagtgcaatatgtaaataagagctatccaaattggaggaaaatcatgatgacgcaaacagcagatacgattttaaataaccccttcttaaataaaggaaccgcgttcacacaagcagaacggcgggaacttggcttggttgggacattgccagcccaagttcaaacgattgatgaacaagccactcaggcctatgcccaataccaaagcaagccaagtgacctggaaaagcggattttcttaatgaatctctttaacgaaaaccggacattattcttccatttaatggatgaacacgtggttgaatt

SEQ ID NO: 7 - DNA, 788 bp, Lactobacillus brevis
ccatacagagccgccctcaacagtttgcagtccttccagcagattctcagcctgcaatcgtgcggcaattcgtggaaaataataattttcgataattggtggcaaccccagcgtggtttggcgagcagctaaatgggctagttcttggtgggctagcgttaattcactgaggacgacttgggcgtgaatggctaattgctcaccgctcggggtaatttgaatatcattgtgtacccgatctcggatgactaatttggtttcaaattcggtctctaatcgtttgatagccgtggtgatcgtgggctgagtcacaccgaagaaggctgctaccttagaaaaatttttttgtagaataagctgctggaaataatccaaatcttttgtattcatattttctcctgtcaaatcaaggctgattactacattataaaataattttataacaatcgctacgtttgactataaaattttcagggcgttatagtgcaatatgtaaataagagctatccaaattggaggaaaatcatgatgacgcaaacagcagatacgattttaaataaccccttcttaaataaaggaaccgcgttcacacaagcagaacggcgggaacttggcttggttgggacattgccagcccaagttcaaacgattgatgaacaagccactcaggcctatgcccaataccaaagcaagccaagtgacctggaaaagcggattttcttaatgaatctctttaacgaaaaccggacattattcttccatttaatggatgaacacgtggttgaatt

SEQ ID NO: 8 - DNA, 788 bp, Lactobacillus brevis
ccatacagagccaccctcaaccgtttgcagtccttccagcagattctcagcctgcaatcgtgcggcaattcgtggaaaataataattttcgataattggtggcaaccccagcgtggtttggcgagcagctaaatgtgctagttcttggtgggctagcgttaattcactgaggacgacttgggcgtgaatggctagttgctcaccgctcggggtaatttgaatatcattgtgtacccgatcccggatgactaatttggtttcaaattcggtctctaatcgtttgatagccgtggtgatcgtgggctgagtcacaccgaagaaggttgctaccttagaaaaatttttttgtagaataagctgctggaaataatccaaatcttttgtattcatattttctcctgtcaaatcaaggctgattgctacattataaaataattttataacaatcgctacatttgactataaaatttccagggcgttatagtgcaatatgtaaataagagctatccaaattggaggaaaatcatgatgacgcaaacagcagatacgattttaaataaccccttcttaaataaaggaaccgcgttcacacaagcagaacggcgggaacttggcttggttgggacattgccagcccaagttcaaacgattgatgaacaagccactcaggcctatgcccaataccaaagcaagccaagtgacctggagaagcggattttcttaatgaatctctttaacgaaaaccggacattattcttccatttaatggatgaacacgtggttgaatt

SEQ ID NO: 9 - DNA, 788 bp, Lactobacillus brevis
ccatacagagccgccctcaacagtttgcagtccttccagcagattctcagcctgcaatcgtgcggcaattcgtggaaaataatagttttcgataattggtggcaaccccagcgtggtttggcgagcagctaaatgggctagttcttggtgggctagcgttaattcactaaggacgacttgggcgtgaatggctaattgctcaccgctcggggtaatttgaatatcattgtgtacccgatcccggatgactaatttggtttcaaattcggtctctaatcgtttgatagccgtggtgatcgtgggctgagtcacaccgaagaaggctgctaccttagaaaaatttttttgtagaataagctgctggaaataatccaaatcttttgtattcatattttctcctgtcaaatcaaggctaattgctacattataaaataattttataacaatcgctacatttgactataaaatttccagggcgttatagtgcaatatgtaaataagagctatccaaattggaggaaaatcatgatgacgcaaacagcagatacgattttaaataaccccttcttaaataaaggaaccgcgttcacgcaagcagaacggcgggaacttggcttggttgggacattgccagcccaagttcaaacgattgatgaacaagccactcaggcctatgctcaataccaaagcaagccaagtgacctggagaagcggattttcttaatgaatctctttaacgaaaaccggacattattcttccatttaatggatgaacatgtggttgaatt

SEQ ID NO: 10 - DNA, 788 bp, Lactobacillus brevis
ccatacagagccgccctcaacagtttgcagtccttccagcagattctcagcctgcaatcgtgcggcaattcgtggaaaataataattttcgataattggtggcaaccccagcgttgtttggcgagcagctaaatgggctagttcttggtgggctagcgttaattcactgaggacgacttgggcgtgaatggctaattgctcaccgctcggggtaatttgaatatcattgtgtacccgatcccggatgactaatttggtttcaaattcggtctctaatcgtttgatagccgtggtgatcgtgggctgagtcacaccgaagaaggctgctaccttagaaaaatttttttgtagaataagctgctggaaataatccaaatcttttgtattcatattttctcctgtcaaatcaaggctgattgctacattataaaataattttataacaatcgctacatttgactataaaatttccagggcgttatagtgcaatatgtaaataagagctatccaaattggaggaaaatcatgatgacgcaaacagcagatacgattttaaataaccccttcttaaataaaggaaccgcgttcacacaagcagaacggcgggaacttggcttggttgggacattgccagcccaagttcaaacgattgatgaacaagccactcaggcctatgcccaataccaaagcaagccaagtgacctggagaagcggattttcttaatgaacctctttaacgaaaaccggacattattcttccatttaatggatgaacatgtggttgaatt

SEQ ID NO: 11 - DNA, 787 bp, Lactobacillus brevis
catacagagccgccctcaacagtttgcagtccttccagcagattctcagcctgcaatcgtgcggcaattcgtggaaaataataattttcgataattggtggcaaccccagcgtggtttggcgagcagctaaatgggctagttcttggtgggctagcgttaattcactgaggacgacttgggcgtgaatggctaattgctcaccgctcggggtaatttgaatatcattgtgtacccgatctcggatgactaatttggtttcaaattcggtctctaatcgtttgatagccgtggtgatcgtgggctgagtcacaccgaagaaggctgctaccttagaaaaatttttttgtagaataagctgctggaaataatccaaatcttttgtattcatattttctcctgtcaaatcaaggctgattactacattataaaataattttataacaatcgctacgtttgactataaaattttcagggcgttatagtgcaatatgtaaataagagctatccaaattggaggaaaatcatgatgacgcaaacagcagatacgattttaaataaccccttcttaaataaaggaaccgcgttcacacaagcagaacggcgggaacttggcttggttgggacattgccagcccaagttcaaacgattgatgaacaagccactcaggcctatgcccaataccaaagcaagccaagtgacctggaaaagcggattttcttaatgaatctctttaacgaaaaccggacattattcttccatttaatggatgaacacgtggttgaatt

SEQ ID NO: 12 - DNA, 26 bp, Oenococcus oeni
  primer_bind 1..26: /note="primer Oenococcus"
aaataataattaccaatgatttgcgg

SEQ ID NO: 13 - DNA, 23 bp, Oenococcus oeni
  primer_bind 1..13: /note="primer Oenococcus"
ataccagttccctgaatatcatc

SEQ ID NO: 14 - DNA, 26 bp, Oenococcus oeni
  primer_bind 1..26: /note="primer Oenococcus"
aartaawaattwccratdatytgcgg

SEQ ID NO: 15 - DNA, 23 bp, Oenococcus oeni
  primer_bind 1..23: /note="primer Oenococcus"
atwccdgtdccytgratatcatc

SEQ ID NO: 16 - DNA, 24 bp, Oenococcus oeni
  primer_bind 1..24: /note="primer Oenococcus"
gtcggttggctgacattgaaaaaa

SEQ ID NO: 17 - DNA, 26 bp, Oenococcus oeni
  primer_bind 1..26: /note="primer Oenococcus"
tttaaaatacctactggatctgtcat

SEQ ID NO: 18 - DNA, 25 bp, Oenococcus oeni
  primer_bind 1..25: /note="primer Oenococcus"
cratyggcatraattcaacmacrtg

SEQ ID NO: 19 - DNA, 23 bp, Lactobacillus
  primer_bind 1..23: /note="primer Lactobacillus"
tcccaygcaatktcytgytksgc

SEQ ID NO: 20 - DNA, 23 bp, Lactobacillus
  primer_bind 1..23: /note="primer Lactobacillus"
  variation 3: /replace="any base"
  variation 6: /replace="any base"
  variation 9: /replace="any base"
  variation 12: /replace="any base"
  variation 21: /replace="any base"
gcngtnccnttntttaaaaangg

SEQ ID NO: 21 - DNA, 23 bp, Lactobacillus
  primer_bind 1..23: /note="primer Lactobacillus"
tcataaacgattggcataaattc

SEQ ID NO: 22 - DNA, 22 bp, Lactobacillus
  primer_bind 1..22: /note="primer Lactobacillus"
cgrtcaaattcttcrgcaatca

SEQ ID NO: 23 - DNA, 11 bp, Bifidobacterium
  misc_feature 1..11: /note="11-mer"
aacacgccaaa

SEQ ID NO: 24 - DNA, 15 bp, Bifidobacterium
  misc_feature 1..15: /note="15-mer"
attggaaggaaagta

SEQ ID NO: 25 - DNA, 10 bp, Bifidobacterium
gagtgctaat

SEQ ID NO: 26 - DNA, 15 bp, Bifidobacterium
attgtattagcactc

SEQ ID NO: 27 - DNA, 1970 bp, Oenococcus alcolitolerans
  LMG_27599_mleA-mleR
tgatcgatctcgtcgtgagcggccaaaatctgcgtaaggatcctttctgtgtacttttcgaggatcttaccggctttcgtcaattgaacgcggccatgcgaatgattcctggtaactaattcttgtttaaattctttttccaatcgctggatggcataagaaatagttggttggctgacattgaaaaaagctgccgtttgtgaaaacgactccactttggccaggcgctgaaaatactctaaatcagtgaatttcatataaatttattttatctcttttgcagcttttgactatatcagctgcgataaaatatcctgaatctgtttgtttattaggagagagaaatgacagatccagtagatattttaaacgatccctttaaaaacaaaggaaccgcttttactcaagaagaacgcaaagcactgggcttgcagggacttttgccctcatgtgtgcaaactattgatcagcaagctgcacaagcctatgctcaatttcaaagcaaagctgataatctagaaaaaagacttttcttgatggaacttttcaacaccaaccacgtgctgttctataagcttttttcacaacacgtcgttgaattcatgccgatcgtctatgatccgactatcgctgatacgattgaaaattattctgaacttttcgttgaaacacagggagctgcttttttggatatccagcatccagaaaacatcgaagccagtttgaaaaatgccgctgacggtcgtgacataaaattgatcgtcgtcactgatgctgagggcattttaggtatcggcgactggggtgttcaaggggtcgatatcgccgttggaaaattgatggtctacaccgtggctgcaggacttgatccaaagagtgtcttgccggtcgtgatcgatgccggaaccaataatcaaaaacttttaaacgatcctttgtatttaggaaaccgttttaaccgtgttcgcggtcaagcttatgatgattttatcgatacttttgttgaaaaatcggaaaatctttttccagatatgtatttgcattgggaagactttgggcgtttgaatgccgcaaatattttgaatagatataaaaataagatcgccacttttaatgatgatatccaaggaaccggtatcgttgtccttgccggcgttttgggtgctttaaaaatttccggtcaaaaattgactgatcaaacttatatgagttttggtgctggaactgccggaatgggtatcgttaaacagcttcatcaggaaatggtccaacagggtctaagcgagcaggaagccaaaaagcatttttatctggttgataagcaaggtctgctctttgatgatgatcctgatctgactccggaacagaagccttttgctgctaaacgcagcgattttgccgatagcgatcggctaactgatcttttatcggctgttaaagctgtcaaaccaactattttagtcggtacttctactcatccgggtgcttttaccaaagaagttgttgaagagatggccaaaaatgcagaccggccggttattttcccgatctccaatccaacgaaattagcagaagcaaaggcagaagatgttttggcttggtctgacggcaaggccttgatcggtacgggtattccggtcgccgatgttgaatataaaggagttgaataccagatcggccaagcaaacaatgccttgatctatccaggcctcggttttggtgctattgccgctgatgccaaattgctgacgcctgagatgatatcagccgctgcacacagtttgggcggaatcgttgatacgcaaaaagccggtgccgcagttttgccgccggtttctaaattggcagaattttcgaaaacggttgctgtggctgtggcccaaaaagctgttgaacagggagttaaccgtcatcctatcagcgatgttaaaaaggcggtagaagatctgaaatgggagcctgaatattaa

SEQ ID NO: 28 - DNA, 17 bp, Lactobacillus brevis
gtraagcgtccyttrtt

SEQ ID NO: 29 - DNA, 17 bp, Lactobacillus brevis
  mlr-Lb-Fc
gtaaygwggytgrstac

SEQ ID NO: 30 - RNA, 17 nt, Lactobacillus brevis
  mlr-Lb-Ft
gtaaygwggytgrstat

SEQ ID NO: 31 - DNA, 21 bp, Lactobacillus brevis
  mleR-cas-F1
gcggtcgtaatgtggtgctac

SEQ ID NO: 32 - DNA, 21 bp, Lactobacillus brevis
  mleR-oen-F1
gcaaaggaaatgtggtgctac

SEQ ID NO: 33 - DNA, 21 bp, Lactobacillus brevis
  mleR-pla-F1
gcggtggtcacgtggtgctac

SEQ ID NO: 34 - DNA, 15 bp, Lactobacillus brevis
  Lb_mleA-R11
gtaaagcgtcctttt

SEQ ID NO: 35 - DNA, 19 bp, Lactobacillus brevis
  mleA_cas_R11
cctggtaaagcgtcctttt

SEQ ID NO: 36 - DNA, 20 bp, Lactobacillus brevis
  mleA_oen-R11
cttccgtaaagcgtcctttt

SEQ ID NO: 37 - DNA, 19 bp, Lactobacillus brevis
  mleA_pla-R11
ctttgtaaagcgtcctttt

SEQ ID NO: 38 - DNA, 20 bp, Lactobacillus brevis
  Lb_mleA-RN
gtaaangcngtnccnttntt

SEQ ID NO: 39 - DNA, 23 bp, Lactobacillus brevis
  mleA_cas-G-R1
gcngtnccnttntttaaaaangg

SEQ ID NO: 40 - DNA, 20 bp, Lactobacillus brevis
  mleA_cas-G-R2
gtnccnttntttaaaaangg

SEQ ID NO: 41 - DNA, 23 bp, Lactobacillus brevis
  mleR_cas-G-F1
tcccaygcaatktcytgytksgc

SEQ ID NO: 42 - DNA, 19 bp, Lactobacillus brevis
  mleR_cas-G-F3
aygcaatktcytgytksgc

SEQ ID NO: 43 - DNA, 23 bp, Lactobacillus brevis
  Lb_bre_mleA-R1_seq
tcataaacgattggcataaattc

SEQ ID NO: 44 - DNA, 20 bp, Lactobacillus brevis
  Lb_bre_mleR-F1_seq
ggctagtggttcaatcgatc

SEQ ID NO: 45 - DNA, 23 bp, Lactobacillus brevis
  Lb_br-pl_mleA-R1_seq
tcataaacgattggcataaattc

SEQ ID NO: 46 - DNA, 22 bp, Lactobacillus brevis
  Lb_br-pl_mleR-F1_seq
cgrtcaaattcttcrgcaatca

SEQ ID NO: 47 - DNA, 26 bp, Lactobacillus brevis
  OE_mleR_F1_seq
aaataataatttccaataatttgcgg

SEQ ID NO: 48 - DNA, 26 bp, Lactobacillus brevis
  OEX_mleR_F1_seq
aaataataattaccaatgatttgcgg

SEQ ID NO: 49 - DNA, 26 bp, Lactobacillus brevis
  OEX_mleR_FN_seq
aartaawaattwccratdatytgcgg

SEQ ID NO: 50 - DNA, 21 bp, Lactobacillus brevis
  OeX_mleR_68-F1
ggttggctgacattgaaaaaa

SEQ ID NO: 51 - DNA, 24 bp, Lactobacillus brevis
  OeX_mleR_68-F2
gtcggttggctgacattgaaaaaa

SEQ ID NO: 52 - DNA, 61 bp, Lactobacillus brevis
  OeX_mleR_68-F1-GC
cgcccggggcgcgccccgggcggggcgggggcacggggcgggttggctgacattgaaaaaa

SEQ ID NO: 53 - DNA, 64 bp, Lactobacillus brevis
  OeX_mleR_68-F2-GC
cgcccggggcgcgccccgggcggggcgggggcacggggcggtcggttggctgacattgaaaaaa

SEQ ID NO: 54 - DNA, 26 bp, Lactobacillus brevis
  OeX_mleA_01-R1
tttaaaatacctactggatctgtcat

SEQ ID NO: 55 - DNA, 66 bp, Lactobacillus brevis
  OeX_mleA_01-R1-GC
cgcccggggcgcgccccgggcggggcgggggcacggggcgtttaaaatacctactggatctgtcat

SEQ ID NO: 56 - DNA, 25 bp, Lactobacillus brevis
  Oen_mleA_244-R1
caattggcataaattcaacaacatg

SEQ ID NO: 57 - DNA, 25 bp, Lactobacillus brevis
  OeX_mleA_244-R1
cgatcggcatgaattcaaccacgtg

SEQ ID NO: 58 - DNA, 25 bp, Lactobacillus brevis
  OeX_mleA_244-RN
cratyggcatraattcaacmacrtg

SEQ ID NO: 59 - DNA, 11 bp, Lactobacillus brevis
  BfX_tkt-hrcA_Stretch_3
aacacgccaaa

SEQ ID NO: 60 - DNA, 15 bp, Lactobacillus brevis
  BfX_tkt-hrcA_Stretch_4
attggaaggaaagta

SEQ ID NO: 61 - DNA, 15 bp, Lactobacillus brevis
  BfX_tkt-hrcA_Stretch_5
attgtattagcactc

SEQ ID NO: 62 - DNA, 15 bp, Lactobacillus brevis
  BcX_hrcA_grpE_Stretch_1
tttgtttttcttctg

SEQ ID NO: 63 - DNA, 15 bp, Lactobacillus brevis
  BcX_hrcA_grpE_Stretch_2
tgtgttcacctccct

SEQ ID NO: 64 - DNA, 20 bp, Lactobacillus brevis
  BfX_hrc_46-FN
tcytcyacmacrgcscgcag

SEQ ID NO: 65 - DNA, 23 bp, Lactobacillus brevis
  BfX_hrc_46-FN2
tartcytcyacvayrgcscgmag

SEQ ID NO: 66 - DNA, 21 bp, Lactobacillus brevis
  BfX_tkt_170-RN
tcrttcggatcgtgcttgatg

SEQ ID NO: 67 - DNA, 21 bp, Lactobacillus brevis
  BfX_tkt_170-RN2
tcrttcggatcrtgcttgatg

SEQ ID NO: 68 - DNA, 25 bp, Lactobacillus brevis
  BcX_hrcA_991-FN1
tcdgaywtgtcwmaagyrytvacaa

SEQ ID NO: 69 - DNA, 25 bp, Lactobacillus brevis
  BcX_hrcA_991-FN2
tcdgacttgtcaaaagcrytvacaa

SEQ ID NO: 70 - DNA, 23 bp, Lactobacillus brevis
  BcX_hrpE_1311-RN1
ttwtcraartchgcytgwasacg

SEQ ID NO: 71 - DNA, 23 bp, Lactobacillus brevis
  BcX_hrpE_1311-RN2
ttttcaaagtcygcytgaacacg

SEQ ID NO: 72 - DNA, 21 bp, Lactobacillus brevis
  BcX_hrcA-grpE_1095-F1
gagggaggtgaacacaatgtc

SEQ ID NO: 73 - DNA, 21 bp, Lactobacillus brevis
  BcX_hrcA-grpE_1120-R1
gacattgtgttcacctccctc

SEQ ID NO: 74 - DNA, 29 bp, Lactobacillus brevis
  Rck_ftsY-01-R1
gagattctttgcgttttaaaaatttaaac

SEQ ID NO: 75 - DNA, 26 bp, Lactobacillus brevis
  Rck_ftsY-85-RN
gttttywgtaaactattttttattcg

SEQ ID NO: 76 - DNA, 25 bp, Lactobacillus brevis
  Rck_ftsY-834-F1
gctgactaaattagatgggactgcc

SEQ ID NO: 77 - DNA, 27 bp, Lactobacillus brevis
  Rck_ftsY-942-FN
tacabgttttytcwgcamaggaatttg

SEQ ID NO: 78 - DNA, 22 bp, Lactobacillus brevis
  Rck_ftsY-947-FN
gttttytcwgcamaggaatttg

SEQ ID NO: 79 - DNA, 19 bp, Lactobacillus brevis
  Rck_rsmD-33-FN
gttttctwcckcgccattg

SEQ ID NO: 80 - DNA, 22 bp, Lactobacillus brevis
  Rck_rubA_145-RN
caaaatcttctttcatkgcacc

SEQ ID NO: 81 - DNA, 24 bp, Lactobacillus brevis
  Rck_rubA-23-RN
cacamagyargcacatatattttc